European Patent Application EP 4 186 976 A1, published May 31, 2023. Title: N-glycosylation mutated rice, method for manufacturing thereof, and method for manufacturing rice for protein production using the same. Applicant: PhytoMab Co., Ltd. The sequence listing filed with the application follows.

SEQUENCE LISTING (45 sequences)

SEQ ID NO: 1 - DNA, 20 bp, Oryza sativa
agagagtatcctcagatcga

SEQ ID NO: 2 - DNA, 20 bp, Oryza sativa
ggcctttgagaattccaacg

SEQ ID NO: 3 - DNA, 20 bp, Oryza sativa
actcctgtgaggggtacttc

SEQ ID NO: 4 - DNA, 20 bp, Oryza sativa
gttaggtaaatccgtgactc

SEQ ID NO: 5 - DNA, 20 bp, Oryza sativa
gtacggcgccaactcgaccg

SEQ ID NO: 6 - DNA, 20 bp, Oryza sativa
cgaccttccaaagttaccca

SEQ ID NO: 7 - DNA, 20 bp, Oryza sativa
tcattcttcgaatggaatat

SEQ ID NO: 8 - DNA, 20 bp, Oryza sativa
ataaaagtatctcatccaca

SEQ ID NO: 9 - DNA, 20 bp, Oryza sativa
gctgccgaggaacttcacct

SEQ ID NO: 10 - DNA, 20 bp, Oryza sativa
tgcctggccatgcagaatca

SEQ ID NO: 11 - DNA, 20 bp, Oryza sativa
gaccgggtagaaattcctgg

SEQ ID NO: 12 - DNA, 20 bp, Oryza sativa
gggtggagcgagcaccagag

SEQ ID NO: 13 - DNA, 20 bp, Oryza sativa
cttgaaggatgccttccaga

SEQ ID NO: 14 - DNA, 20 bp, Oryza sativa
atgccaacgtcggtgagcca

SEQ ID NO: 15 - DNA, 20 bp, Oryza sativa
aggggagcgtcgtcgaggtg

SEQ ID NO: 16 - DNA, 20 bp, Oryza sativa
ttactcagagagatatacaa

SEQ ID NO: 17 - DNA, 22 bp, Artificial Sequence
  a1,3-FucT-F T1
ccctcaagctttatgctcaact

SEQ ID NO: 18 - DNA, 21 bp, Artificial Sequence
  a1,3-FucT-R T1
gttccgtagctggggatacat

SEQ ID NO: 19 - DNA, 21 bp, Artificial Sequence
  a1,3-FucT-F_T2
ttgttttggacattgatgcac

SEQ ID NO: 20 - DNA, 20 bp, Artificial Sequence
  a1,3-FucT-R_T2
ttccaccccagagagatgac

SEQ ID NO: 21 - DNA, 21 bp, Artificial Sequence
  b1,2-XylT-F_T1
caccacaacaacagcaacaac

SEQ ID NO: 22 - DNA, 20 bp, Artificial Sequence
  b1,2-XylT-R_T1
gtacttgggcagctcctcct

SEQ ID NO: 23 - DNA, 24 bp, Artificial Sequence
  b1,2-XylT-F_T2
cctattgttatattgcaggattca

SEQ ID NO: 24 - DNA, 25 bp, Artificial Sequence
  b1,2-XylT-R_T2
gaatcacattataaaggagcgaagg

SEQ ID NO: 25 - DNA, 21 bp, Artificial Sequence
  b1,3-Gal-R_T1
tgcagttcagaatccacagaa

SEQ ID NO: 26 - DNA, 20 bp, Artificial Sequence
  b1,3-Gal-R_T1
aagcacaattggagggtctg

SEQ ID NO: 27 - DNA, 20 bp, Artificial Sequence
  b1,3-Gal-F_T2
ccatctgcatctatggggta

SEQ ID NO: 28 - DNA, 24 bp, Artificial Sequence
  b1,3-Gal-R_T2
tgatggtgcacacaataacttaaa

SEQ ID NO: 29 - DNA, 20 bp, Artificial Sequence
  a1,4-FucT-F_T1
ctcccaccctttccactgta

SEQ ID NO: 30 - DNA, 19 bp, Artificial Sequence
  a1,4-FucT-R_T1
acgtgtacaccccgtcgag

SEQ ID NO: 31 - DNA, 20 bp, Artificial Sequence
  a1,4-FucT-F_T2
tcttcactgcgcaatgtcac

SEQ ID NO: 32 - DNA, 21 bp, Artificial Sequence
  a1,4-FucT-R_T2
gccacaaaaatatcacctcgt

SEQ ID NO: 33 - DNA, 20 bp, Artificial Sequence
  Hexo1-F_T1 primer
atacccgggcacatttacag

SEQ ID NO: 34 - DNA, 20 bp, Artificial Sequence
  Hexo1-R_T1 primer
ccactccaagctccagctac

SEQ ID NO: 35 - DNA, 20 bp, Artificial Sequence
  Hexo2-F_T1 primer
cgacgagtcctacacgctct

SEQ ID NO: 36 - DNA, 19 bp, Artificial Sequence
  Hexo2-R_T1 primer
gagtaggagccggagttgg

SEQ ID NO: 37 - DNA, 22 bp, Artificial Sequence
  Hexo3-F_T1 primer
cattacgaaatggcttttccat

SEQ ID NO: 38 - DNA, 22 bp, Artificial Sequence
  Hexo3-R_T1 primer
tgctattcaacaggccaagtta

SEQ ID NO: 39 - DNA, 22 bp, Artificial Sequence
  Hexo4-F_T1 primer
ggcgtttctcttcatcttcttg

SEQ ID NO: 40 - DNA, 20 bp, Artificial Sequence
  Hexo4-R_T1 primer
cagctctatcagcgtcacca

SEQ ID NO: 41 - protein, 214 aa, Unknown
  trastuzumab light chain
DIQMTQSPSSLSASVGDRVTITCRASQDVNTAVAWYQQKPGKAPKLLIYSASFLYSGVPSRFSGSRSGTDFTLTISSLQPEDFATYYCQQHYTTPPTFGQGTKVEIKRTVAAPSVFIFPPSDEQLKSGTASVVCLLNNFYPREAKVQWKVDNALQSGNSQESVTEQDSKDSTYSLSSTLTLSKADYEKHKVYACEVTHQGLSSPVTKSFNRGEC

SEQ ID NO: 42 - protein, 450 aa, Unknown
  trastuzumab heavy chain
EVQLVESGGGLVQPGGSLRLSCAASGFNIKDTYIHWVRQAPGKGLEWVARIYPTNGYTRYADSVKGRFTISADTSKNTAYLQMNSLRAEDTAVYYCSRWGGDGFYAMDYWGQGTLVTVSSASTKGPSVFPLAPSSKSTSGGTAALGCLVKDYFPEPVTVSWNSGALTSGVHTFPAVLQSSGLYSLSSVVTVPSSSLGTQTYICNVNHKPSNTKVDKKVEPKSCDKTHTCPPCPAPELLGGPSVFLFPPKPKDTLMISRTPEVTCVVVDVSHEDPEVKFNWYVDGVEVHNAKTKPREEQYNSTYRVVSVLTVLHQDWLNGKEYKCKVSNKALPAPIEKTISKAKGQPREPQVYTLPPSREEMTKNQVSLTCLVKGFYPSDIAVEWESNGQPENNYKTTPPVLDSDGSFFLYSKLTVDKSRWQQGNVFSCSVMHEALHNHYTQKSLSLSPGK

SEQ ID NO: 43 - protein, 24 aa, Oryza sativa
GKHHVTLCCVVFAVLCLASSLAQA

SEQ ID NO: 44 - DNA, 723 bp, Artificial Sequence
  trastuzumab light chain
atgggcaagcaccacgtgaccctgtgctgcgtggtgtttgctgttctgtgcctggcaagcagcctggcacaggcagacatccagatgacacagagccctagcagcctgagcgcatctgtgggcgatcgcgtgacaattacatgccgcgcaagccaggacgtgaacaccgcagttgcatggtaccagcagaagccaggcaaggccccaaagctgctgatctacagcgccagcttcctgtacagcggcgtgccatctcgctttagcggttctcgcagcggcaccgatttcaccctgacaatctctagcctgcagccagaggacttcgccacctactactgccagcagcactacaccacaccaccaacattcggccagggcaccaaggtcgagatcaagcgaacagtggcagccccaagcgtgttcatcttcccaccatctgacgagcagctgaagtccggcacagcttctgtggtgtgcctgctgaacaacttctacccacgcgaggccaaggtgcagtggaaggttgacaacgcactgcagagcggcaacagccaggagagcgttacagagcaggacagcaaggactccacctacagcctgtccagcacactgaccctgagcaaggccgactacgagaagcacaaggtgtacgcctgcgaggtgacacaccagggcctgtcatctccagtgaccaagtctttcaaccgcggcgagtgctgatga

SEQ ID NO: 45 - DNA, 1431 bp, Artificial Sequence
  trastuzumab heavy chain
atgggcaagcaccacgtgaccctgtgctgcgtggtgtttgctgttctgtgcctggcaagcagcctggcacaggcagaggttcagctggttgagtctggcggtggtctggttcagcctggtggttctctgcgactgtcttgcgcagcaagcggcttcaacatcaaggacacctacatccactgggtgcgccaggcaccaggtaagggcctggagtgggttgcacgcatctaccctaccaacggctacacccgctacgccgattctgtgaagggccgctttaccatcagcgccgacaccagcaagaacaccgcctacctgcagatgaacagcctgcgcgctgaggacaccgcagtgtactactgctctcgatggggcggtgacggcttctacgcaatggattactggggccagggcaccctggtgacagtgtctagcgcatctacaaagggcccaagcgtgttcccactggcaccaagcagcaagtctacaagcggcggtacagcagcactgggctgcctggtgaaggactactttccagagccagtgaccgtgagctggaacagcggtgcactgacatctggcgtgcacacattcccagcagtgctgcagtcaagcggcctgtactctctgagcagcgtggtgaccgtgccatcttcttcactgggcacccagacctacatctgcaacgtgaaccacaagccaagcaacaccaaggtggacaagaaggtcgagccaaagagctgcgacaagacccacacatgcccaccatgccctgcaccagagctgctcggtggcccatctgtgtttctgttcccaccaaagccaaaggacaccctgatgatcagccgcacaccagaggtgacatgcgtggtggtggatgtgagccacgaggaccctgaggtgaagttcaactggtacgtggacggcgtcgaggtgcacaacgcaaagacaaagccacgcgaggagcagtacaacagcacctaccgagtggtgtccgtgctcactgtgctgcaccaggattggctgaacggcaaggagtacaagtgcaaggtgagcaacaaggccctgccagcaccaatcgagaagaccatcagcaaggccaagggccagccacgagagccacaggtttacaccctgccaccatctcgcgaggagatgaccaagaaccaggtgagcctgacctgcctcgtcaagggcttctacccaagcgacattgccgtcgagtgggagtctaacggccagcctgagaacaactacaagaccacaccaccagtgctggacagcgacggctcattcttcctgtacagcaagctgaccgtggacaagtcccgatggcagcagggcaacgtgttcagctgctctgtgatgcacgaggccctgcacaaccactacacccagaagtccctgagcctgtctccaggcaagtgatga